European Patent Application EP 4 269 568 A1, published November 1, 2023. Title: PREPARATION METHOD FOR TUMOR-INFILTRATING LYMPHOCYTE AND USE THEREOF. Applicant: Suzhou Grit Biotechnology Co., Ltd.; Shanghai Grit Biotechnology Co., Ltd.; Zhuhai Tuoyu Biotechnology Co., Ltd.; Zhuhai Grit Biotechnology Co., Ltd. The sequence listing filed with the application follows.

SEQUENCE LISTING (33 sequences)

SEQ ID NO: 1 - protein, 8 aa, Artificial Sequence
  OKT3 HCDR1
GYTFTRYT

SEQ ID NO: 2 - protein, 8 aa, Artificial Sequence
  OKT3 HCDR2
INPSRGYT

SEQ ID NO: 3 - protein, 12 aa, Artificial Sequence
  OKT3 HCDR3
ARYYDDHYSLDY

SEQ ID NO: 4 - protein, 5 aa, Artificial Sequence
  OKT3 LCDR1
SSVSY

SEQ ID NO: 5 - protein, 3 aa, Artificial Sequence
  OKT3 LCDR2
DTS

SEQ ID NO: 6 - protein, 9 aa, Artificial Sequence
  OKT3 LCDR3
QQWSSNPFT

SEQ ID NO: 7 - protein, 119 aa, Artificial Sequence
  OKT3 variable heavy chain VH
QVQLVQSGGGVVQPGRSLRLSCKASGYTFTRYTMHWVRQAPGKGLEWIGYINPSRGYTNYNQKVKDRFTISRDNSKNTAFLQMDSLRPEDTGVYFCARYYDDHYSLDYWGQGTPVTVSS

SEQ ID NO: 8 - protein, 106 aa, Artificial Sequence [sequence omitted]

SEQ ID NO: 9 - protein, 222 aa, Artificial Sequence
  OKT3 heavy chain
QVQLVQSGGGVVQPGRSLRLSCKASGYTFTRYTMHWVRQAPGKGLEWIGYINPSRGYTNYNQKVKDRFTISRDNSKNTAFLQMDSLRPEDTGVYFCARYYDDHYSLDYWGQGTPVTVSSASTKGPSVFPLAPSSKSTSGGTAALGCLVKDYFPEPVTVSWNSGALTSGVHTFPAVLQSSGLYSLSSVVTVPSSSLGTQTYICNVNHKPSNTKVDKKVEPKSC

SEQ ID NO: 10 - protein, 213 aa, Artificial Sequence
  OKT3 light chain
DIQMTQSPSSLSASVGDRVTITCSASSSVSYMNWYQQTPGKAPKRWIYDTSKLASGVPSRFSGSGSGTDYTFTISSLQPEDIATYYCQQWSSNPFTFGQGTKLQITRTVAAPSVFIFPPSDEQLKSGTASVVCLLNNFYPREAKVQWKVDNALQSGNSQESVTEQDSKDSTYSLSSTLTLSKADYEKHKVYACEVTHQGLSSPVTKSFNRGEC

SEQ ID NO: 11 - protein, 5 aa, Artificial Sequence
  SP34 HCDR1
TYAMN

SEQ ID NO: 12 - protein, 19 aa, Artificial Sequence
  SP34 HCDR2
RIRSKYNNYATYYADSVKD

SEQ ID NO: 13 - protein, 14 aa, Artificial Sequence
  SP34 HCDR3
HGNFGNSYVSWFAY

SEQ ID NO: 14 - protein, 14 aa, Artificial Sequence
  SP34 LCDR1
RSSTGAVTTSNYAN

SEQ ID NO: 15 - protein, 7 aa, Artificial Sequence
  SP34 LCDR2
GTNKRAP

SEQ ID NO: 16 - protein, 9 aa, Artificial Sequence
  SP34 LCDR3
ALWYSNLWV

SEQ ID NO: 17 - protein, 125 aa, Artificial Sequence
  SP34 variable heavy chain VH
EVQLVESGGGLVQPKGSLKLSCAASGFTFNTYAMNWVRQAPGKGLEWVARIRSKYNNYATYYADSVKDRFTISRDDSQSILYLQMNNLKTEDTAMYYCVRHGNFGNSYVSWFAYWGQGTLVTVSS

SEQ ID NO: 18 - protein, 109 aa, Artificial Sequence
  SP34 variable light chain VL
QAVVTQESALTTSPGETVTLTCRSSTGAVTTSNYANWVQEKPDHLFTGLIGGTNKRAPGVPARFSGSLIGDKAALTITGAQTEDEAIYFCALWYSNLWVFGGGTKLTVL

SEQ ID NO: 19 - protein, 228 aa, Artificial Sequence
  SP34 heavy chain
EVQLVESGGGLVQPKGSLKLSCAASGFTFNTYAMNWVRQAPGKGLEWVARIRSKYNNYATYYADSVKDRFTISRDDSQSILYLQMNNLKTEDTAMYYCVRHGNFGNSYVSWFAYWGQGTLVTVSSASTKGPSVFPLAPSSKSTSGGTAALGCLVKDYFPEPVTVSWNSGALTSGVHTFPAVLQSSGLYSLSSVVTVPSSSLGTQTYICNVNHKPSNTKVDKKVEPKSC

SEQ ID NO: 20 - protein, 216 aa, Artificial Sequence
  SP34 light chain
QAVVTQESALTTSPGETVTLTCRSSTGAVTTSNYANWVQEKPDHLFTGLIGGTNKRAPGVPARFSGSLIGDKAALTITGAQTEDEAIYFCALWYSNLWVFGGGTKLTVLRTVAAPSVFIFPPSDEQLKSGTASVVCLLNNFYPREAKVQWKVDNALQSGNSQESVTEQDSKDSTYSLSSTLTLSKADYEKHKVYACEVTHQGLSSPVTKSFNRGEC

SEQ ID NO: 21 - protein, 8 aa, Artificial Sequence
  15E8 HCDR1
GFSLTSYG

SEQ ID NO: 22 - protein, 7 aa, Artificial Sequence
  15E8 HCDR2
IWAGGST

SEQ ID NO: 23 - protein, 17 aa, Artificial Sequence
  15E8 HCDR3
ARDKRAPGKLYYGYPDY

SEQ ID NO: 24 - protein, 10 aa, Artificial Sequence
  15E8 LCDR1
ESVEYYVTSL

SEQ ID NO: 25 - protein, 3 aa, Artificial Sequence
  15E8 LCDR2
AAS

SEQ ID NO: 26 - protein, 9 aa, Artificial Sequence
  15E8 LCDR3
QQTRKVPST

SEQ ID NO: 27 - protein, 123 aa, Artificial Sequence
  15E8 variable heavy chain VH 1
QVQLQESGPGLVKPSETLSLTCTVSGFSLTSYGVHWIRQPPGKGLEWLGVIWAGGSTNYNSSLKSRVTISKDTSKNQVFLKLSSVTADDTAVYYCARDKRAPGKLYYGYPDYWGQGTTLTVSS

SEQ ID NO: 28 - protein, 123 aa, Artificial Sequence
  15E8 variable heavy chain VH 2
QVQLQESGPGLVKPSETLSLTCTVSGFSLTSYGVHWIRQPPGKGLEWLGVIWAGGSTNYNSSLKSRVTISKDTSKNQVSLKLSSVTAADTAVYYCARDKRAPGKLYYGYPDYWGQGTTLTVSS

SEQ ID NO: 29 - protein, 111 aa, Artificial Sequence
  15E8 variable light chain VL
DIVMTQSPDSLAVSLGERATINCRASESVEYYVTSLMQWYQQKPGQPPKLLIYAASNVESGVPARFSGSGSGTDFTLTISPLQAEDVAVYYCQQTRKVPSTFGGGTKLEIK

SEQ ID NO: 30 - protein, 226 aa, Artificial Sequence
  15E8 heavy chain  1
QVQLQESGPGLVKPSETLSLTCTVSGFSLTSYGVHWIRQPPGKGLEWLGVIWAGGSTNYNSSLKSRVTISKDTSKNQVFLKLSSVTADDTAVYYCARDKRAPGKLYYGYPDYWGQGTTLTVSSASTKGPSVFPLAPSSKSTSGGTAALGCLVKDYFPEPVTVSWNSGALTSGVHTFPAVLQSSGLYSLSSVVTVPSSSLGTQTYICNVNHKPSNTKVDKKVEPKSC

SEQ ID NO: 31 - protein, 226 aa, Artificial Sequence
  15E8 heavy chain  2
QVQLQESGPGLVKPSETLSLTCTVSGFSLTSYGVHWIRQPPGKGLEWLGVIWAGGSTNYNSSLKSRVTISKDTSKNQVSLKLSSVTAADTAVYYCARDKRAPGKLYYGYPDYWGQGTTLTVSSASTKGPSVFPLAPSSKSTSGGTAALGCLVKDYFPEPVTVSWNSGALTSGVHTFPAVLQSSGLYSLSSVVTVPSSSLGTQTYICNVNHKPSNTKVDKKVEPKSC

SEQ ID NO: 32 - protein, 218 aa, Artificial Sequence
  15E8 light chain
DIVMTQSPDSLAVSLGERATINCRASESVEYYVTSLMQWYQQKPGQPPKLLIYAASNVESGVPARFSGSGSGTDFTLTISPLQAEDVAVYYCQQTRKVPSTFGGGTKLEIKRTVAAPSVFIFPPSDEQLKSGTASVVCLLNNFYPREAKVQWKVDNALQSGNSQESVTEQDSKDSTYSLSSTLTLSKADYEKHKVYACEVTHQGLSSPVTKSFNRGEC

SEQ ID NO: 33 - DNA, 20 bp, Artificial Sequence
  TCRbeta sgRNA
ggagaatgacgagtggaccc